European Patent Application EP 4 509 135 A2, published February 19, 2025. Title: ENGINEERED DNASE ENZYMES AND USE IN THERAPY. Applicant: Neutrolis, Inc. Application EP. The sequence listing filed with the application follows.

SEQUENCE LISTING (40 sequences)

SEQ ID NO: 1 - protein, 282 aa, Homo sapiens [sequence omitted]

SEQ ID NO: 2 - protein, 305 aa, Homo sapiens
MSRELAPLLLLLLSIHSALAMRICSFNVRSFGESKQEDKNAMDVIVKVIKRCDIILVMEIKDSNNRICPILMEKLNRNSRRGITYNYVISSRLGRNTYKEQYAFLYKEKLVSVKRSYHYHDYQDGDADVFSREPFVVWFQSPHTAVKDFVIIPLHTTPETSVKEIDELVEVYTDVKHRWKAENFIFMGDFNAGCSYVPKKAWKNIRLRTDPRFVWLIGDQEDTTVKKSTNCAYDRIVLRGQEIVSSVVPKSNSVFDFQKAYKLTEEEALDVSDHFPVEFKLQSSRAFTNSKKSVTLRKKTKSKRS

SEQ ID NO: 3 - protein, 284 aa, Mus musculus
MRYTGLMGTLLTLVNLLQLAGTLRIAAFNIRTFGETKMSNATLSVYFVKILSRYDIAVIQEVRDSHLVAVGKLLDELNRDKPDTYRYVVSEPLGRKSYKEQYLFVYRPDQVSILDSYQYDDGCEPCGNDTFSREPAIVKFFSPYTEVQEFAIVPLHAAPTEAVSEIDALYDVYLDVWQKWGLEDIMFMGDFNAGCSYVTSSQWSSIRLRTSPIFQWLIPDSADTTVTSTHCAYDRIVVAGALLQAAVVPNSAVPFDFQAEYGLSNQLAEAISDHYPVEVTLRKI

SEQ ID NO: 4 - protein, 284 aa, synthetic construct
  REGION 1..284: note = Artificial synthetic polypeptide sequence
MRYTGLMGILLTLVNLLQLAATLRIAAFNIRTFGDTKMSNATLSSYIVKILSRYDIAVVQEVRDTHLVAVGKLLDELNRDIPDNYRYIISEPLGRKSYKEQYLFVYRPSQVSVLDSYHYDDGCEPCGNDTFSREPAIVKFFSPYTEVREFAIVPLHSAPTEAVSEIDALYDVYLDVRQKWGLEDIMFMGDFNAGCSYVTSSQWSSIRLRTSPIFQWLIPDSADTTATSTHCAYDRIVVAGALLQAAVVPSSAVPFDFQAEYRLTNQMAEAISDHYPVEVTLRKT

SEQ ID NO: 5 - protein, 282 aa, synthetic construct
  REGION 1..282: note = Artificial synthetic polypeptide sequence
MRGMKLLGALLALAALLQGAVSLKIAAFNIRTFGETKMSNATLVSYIVKILSRYDIALVQEVRDSHLTAVGKLLDNLNRDAPDTYHYVVSEPLGRNSYKERYLFVYRPDQVSAVDSYYYDDGCEPCGNDTFNREPAIVRFFSRFTEVREFAIVPLHAAPGDAVAEIDALYDVYLDVQEKWGLEDVMLMGDFNAGCSYVRPSQWSSIRLRTSPTFQWLIPDSADTTATPTHCAYDRIVVAGMLLRGAVVPDSALPFNFQAAYGLSDQLAQAISDHYPVEVMLK

SEQ ID NO: 6 - protein, 282 aa, synthetic construct
  REGION 1..282: note = Artificial synthetic polypeptide sequence
MRGMKLLGALLALAALLQGAVSLKIAAFNIRTFGETKMSNATLVSYIVKILSRYDIALVQEVRDSHLTAVGKLLDNLNRDAPDTYHYVVSEPLGRNSYKERYLFVYRPDQVSAVDSYYYDDGCEPCGNDTFNREPAIVRFFSRFTEVREFAIVPLHAAPGDAVAEIDALYDVYLDVKEKWGLEDVMLMGDFNAGCSYVRPSQWSSIRLRTSPTFQWLIPDSADTTATPTHCAYDRIVVAGMLLRGAVVPDSALPFNFQAAYKLSDQLAQAISDHYPVEVMLK

SEQ ID NO: 7 - protein, 282 aa, synthetic construct
  REGION 1..282: note = Artificial synthetic polypeptide sequence
MRGMKLLGALLALAALLQGAVSLKIAAFNIRTFGETKMSNATLVSYIVQILSRYDIALVQEVRDSHLTAVGKLLDNLNQDAPDTYHYVVSEPLGRNSYKERYLFVYRPDQVSAVDSYYYDDGCEPCGNDTFNREPFIVRFFSRFTEVREFAIVPLHAAPGDAVAEIDALYDVYLDVQEKWGLEDVMLMGDFNAGCSYVRPSQWSSIRLWTSPTFQWLIPDSADTTAKPTHCAYDRIVVAGMLLRGAVVPDSALPFNFQAAYGLSDQLAQAISDHYPVEVMLK

SEQ ID NO: 8 - protein, 282 aa, synthetic construct
  REGION 1..282: note = Artificial synthetic polypeptide sequence
MRGMKLLGALLALAALLQGAVSLKIAAFNIRTFGETKMSNATLVSYIVQILSRYDIALVQEVRDSHLTAVGKLLDNLNQDAPDTYHYVVSEPLGRNSYKERYLFVYRPDQVSAVDSYYYDDGCEPCGNDTFNREPAIVRFFSRFTEVREFAIVPLHAAPGDAVAEIDALYDVYLDVQEKWGLEDVMLMGDFNAGCSYVRPSQWSSIRLWTSPTFQWLIPDSADTTAKPTHCAYDRIVVAGMLLRGAVVPDSALPFNFQAAYGLSDQLAQAISDHYPVEVMLK

SEQ ID NO: 9 - protein, 282 aa, synthetic construct
  REGION 1..282: note = Artificial synthetic polypeptide sequence
MRGMKLLGALLALAALLQGAVSLKIAAFNIQTFGETKMSNATLVSYIVQILSRYDIALVQEVRDSHLTAVGKLLDNLNQDAPDTYHYVVSEPLGRNSYKERYLFVYRPDQVSAVDSYYYDDGCEPCGNDTFNREPFIVRFFSRFTEVREFAIVPLHAAPGDAVKEIDALYDVYLDVQEKWGLEDVMLMGDFNAGCSYVRPSQWSSIRLWTSPTFQWLIPDSADTTATPTHCAYDRIVVAGMLLRGAVVPDSALPFNFQAAYGLSDQLAQAISDHYPVEVMLK

SEQ ID NO: 10 - protein, 284 aa, synthetic construct
  REGION 1..284: note = Artificial synthetic polypeptide sequence
MRGMKLLGALLALAALLQGAVSLKIAAFNIQTFGETKMSNATLVSYIVQILSRYDIALVQEVRDSHLTAVGKLLDNLNRNSRRGITYHYVVSEPLGRNSYKERYLFVYRPDQVSAVDSYYYDDGCEPCGNDTFNREPAIVRFFSRFTEVREFAIVPLHAAPGDAVAEIDALYDVYLDVQEKWGLEDVMLMGDFNAGCSYVRPSQWSSIRLWTSPTFQWLIPDSADTTATPTHCAYDRIVVAGMLLRGAVVPDSALPFNFQAAYGLSDQLAQAISDHYPVEVMLK

SEQ ID NO: 11 - protein, 282 aa, synthetic construct
  REGION 1..282: note = Artificial synthetic polypeptide sequence
MRGMKLLGALLALAALLQGAVSLKIAAFNIQTFGETKMSNATLVSYIVQILSRYDIALVQEVRDSHLTAVGKLLDNLNQDAPDTYNYVISSRLGRNSYKERYLFVYRPDQVSAVDSYYYDDGCEPCGNDTFNREPAIVRFFSRFTEVREFAIVPLHAAPGDAVAEIDALYDVYLDVQEKWGLEDVMLMGDFNAGCSYVRPSQWSSIRLWTSPTFQWLIPDSADTTATPTHCAYDRIVVAGMLLRGAVVPDSALPFNFQAAYGLSDQLAQAISDHYPVEVMLK

SEQ ID NO: 12 - protein, 282 aa, synthetic construct
  REGION 1..282: note = Artificial synthetic polypeptide sequence
MRGMKLLGALLALAALLQGAVSLKIAAFNIQTFGETKMSNATLVSYIVQILSRYDIALVQEVRDSHLTAVGKLLDNLNQDAPDTYHYVVSEPLGRNSYKERYLFVYRPDQVSAVDSYYYDDGCEPCGNDTFNREPFVVRFFSRFTEVREFAIVPLHAAPGDAVAEIDALYDVYLDVQEKWGLEDVMLMGDFNAGCSYVRPSQWSSIRLWTSPTFQWLIPDSADTTATPTHCAYDRIVVAGMLLRGAVVPDSALPFNFQAAYGLSDQLAQAISDHYPVEVMLK

SEQ ID NO: 13 - protein, 282 aa, synthetic construct
  REGION 1..282: note = Artificial synthetic polypeptide sequence
MRGMKLLGALLALAALLQGAVSLKIAAFNIQTFGETKMSNATLVSYIVQILSRYDIALVQEVRDSHLTAVGKLLDNLNQDAPDTYHYVVSEPLGRNSYKERYLFVYRPDQVSAVDSYYYDDGCEPCGNDTFNREPAIVRFFSRFTEVREFAIVPLHAAPGDAVAEIDALYDVYLDVQEKWGLEDVMLMGDFNAGCSYVPKKAWKNIRLRTDPRFVWLIGDQEDTTATPTHCAYDRIVVAGMLLRGAVVPDSALPFNFQAAYGLSDQLAQAISDHYPVEVMLK

SEQ ID NO: 14 - protein, 283 aa, synthetic construct
  REGION 1..283: note = Artificial synthetic polypeptide sequence
MRGMKLLGALLALAALLQGAVSLKIAAFNIQTFGETKMSNATLVSYIVQILSRYDIALVQEVRDSHLTAVGKLLDNLNQDAPDTYHYVVSEPLGRNSYKERYLFVYRPDQVSAVDSYYYDDGCEPCGNDTFNREPAIVRFFSRFTEVREFAIVPLHAAPGDAVAEIDALYDVYLDVQEKWGLEDVMLMGDFNAGCSYVRPSQWSSIRLWTSPTFQWLIPDSADTTVKKSTHCAYDRIVVAGMLLRGAVVPDSALPFNFQAAYGLSDQLAQAISDHYPVEVMLK

SEQ ID NO: 15 - protein, 285 aa, synthetic construct
  REGION 1..285: note = Artificial synthetic polypeptide sequence
MRGMKLLGALLALAALLQGAVSLKIAAFNIQTFGETKMSNATLVSYIVQILSRYDIALVQEVRDSHLTAVGKLLDNLNRNSRRGITYNYVISSRLGRNSYKERYLFVYRPDQVSAVDSYYYDDGCEPCGNDTFNREPFVVRFFSRFTEVREFAIVPLHAAPGDAVAEIDALYDVYLDVQEKWGLEDVMLMGDFNAGCSYVPKKAWKNIRLRTDPRFVWLIGDQEDTTVKKSTHCAYDRIVVAGMLLRGAVVPDSALPFNFQAAYGLSDQLAQAISDHYPVEVMLK

SEQ ID NO: 16 - protein, 305 aa, synthetic construct
  REGION 1..305: note = Artificial synthetic polypeptide sequence
MRGMKLLGALLALAALLQGAVSLKIAAFNIQTFGETKMSNATLVSYIVQILSRYDIALVQEVRDSHLTAVGKLLDNLNQDAPDTYHYVVSEPLGRNSYKERYLFVYRPDQVSAVDSYYYDDGCEPCGNDTFNREPAIVRFFSRFTEVREFAIVPLHAAPGDAVAEIDALYDVYLDVQEKWGLEDVMLMGDFNAGCSYVRPSQWSSIRLWTSPTFQWLIPDSADTTATPTHCAYDRIVVAGMLLRGAVVPDSALPFNFQAAYGLSDQLAQAISDHFPVEFKLQSSRAFTNSKKSVTLRKKTKSKRS

SEQ ID NO: 17 - protein, 282 aa, synthetic construct
  REGION 1..282: note = Artificial synthetic polypeptide sequence
MSRELAPLLLLLLSIHSALAMRICSFNVRSFGESKQEDKNAMDVIVKVIKRCDIILVMEIKDSNNRICPILMEKLNRNSRRGITYNYVISSRLGRNTYKEQYAFLYKEKLVSVKRSYHYHDYQDGDADVFSREPFVVWFQSPHTAVKDFVIIPLHTTPETSVKEIDELVEVYTDVKHRWKAENFIFMGDFNAGCSYVPKKAWKNIRLRTDPRFVWLIGDQEDTTVKKSTNCAYDRIVLRGQEIVSSVVPKSNSVFDFQKAYKLTEEEALDVSDHYPVEVMLK

SEQ ID NO: 18 - protein, 305 aa, synthetic construct
  REGION 1..305: note = Artificial synthetic polypeptide sequence
MSRELAPLLLLLLSIHSALAMRICSFNVRSFGESKQENKTAMDVIVKVIKRCDIILVMEIKDSNNRICPILMEKLNRNSRRGITYNYVISSRLGRNTYKEQYAFLYKEKLVSVKRSYHYHDYQDGDNDTFSREPFVVWFQSPHTAVKDFVIIPLHTTPETSVKEIDELVEVYTDVKHRWKAENFIFMGDFNAGCSYVPKKAWKNIRLRTDPRFVWLIGDQEDTTVKKSTNCAYDRIVLRGQEIVSSVVPKSNSVFDFQKAYKLTEEEALDVSDHFPVEFKLQSSRAFTNSKKSVTLRKKTKSKRS

SEQ ID NO: 19 - protein, 305 aa, synthetic construct
  REGION 1..305: note = Artificial synthetic polypeptide sequence
MSRELAPLLLLLLSIHSALAMRICSFNVRSFGESKMSNATLVSYIVKVIKRCDIILVMEIKDSNNRICPILMEKLNRNSRRGITYNYVISSRLGRNTYKEQYAFLYKEKLVSVKRSYHYHDYQDGDADVFSREPFVVWFQSPHTAVKDFVIIPLHTTPETSVKEIDELVEVYTDVKHRWKAENFIFMGDFNAGCSYVPKKAWKNIRLRTDPRFVWLIGDQEDTTVKKSTNCAYDRIVLRGQEIVSSVVPKSNSVFDFQKAYKLTEEEALDVSDHFPVEFKLQSSRAFTNSKKSVTLRKKTKSKRS

SEQ ID NO: 20 - protein, 306 aa, synthetic construct
  REGION 1..306: note = Artificial synthetic polynucleotide sequence
MSRELAPLLLLLLSIHSALAMRICSFNVRSFGESKQEDKNAMDVIVKVIKRCDIILVMEIKDSNNRICPILMEKLNRNSRRGITYNYVISSRLGRNTYKEQYAFLYKEKLVSVKRSYHYHDGCEPCGNDTFNREPFVVWFQSPHTAVKDFVIIPLHTTPETSVKEIDELVEVYTDVKHRWKAENFIFMGDFNAGCSYVPKKAWKNIRLRTDPRFVWLIGDQEDTTVKKSTNCAYDRIVLRGQEIVSSVVPKSNSVFDFQKAYKLTEEEALDVSDHFPVEFKLQSSRAFTNSKKSVTLRKKTKSKRS

SEQ ID NO: 21 - protein, 282 aa, synthetic construct
  REGION 1..282: note = Artificial synthetic polypeptide sequence
MRGMKLLGALLALAALLQGAVSLKIAAFNIQTFGETKMSSATLVSYIVQILSRYDIALVQEVRDSHLTAVGKLLDNLNQDAPDTYHYVVSEPLGRNSYKERYLFVYRPDQVSAVDSYYYDDGCEPCGSDTFNREPAIVRFFSRFTEVREFAIVPLHAAPGDAVAEIDALYDVYLDVQEKWGLEDVMLMGDFNAGCSYVRPSQWSSIRLWTSPTFQWLIPDSADTTATPTHCAYDRIVVAGMLLRGAVVPDSALPFNFQAAYGLSDQLAQAISDHYPVEVMLK

SEQ ID NO: 22 - DNA, 846 bp, synthetic construct
  misc_feature 1..846: note = Artificial synthetic polynucleotide sequence
  source 1..846: mol_type = other DNA
atgagaggtatgaagctccttggtgccctcctggctctcgctgctctcctccaaggagcagtttctctaaagattgctgctttcaatattcaaacctttggcgagactaaaatgtcctcggcaacattagtatcttacattgttcagatcctttctcgttacgacatagctttggtccaggaggttagagactcccacttgactgccgtcggtaagctgctagacaatcttaaccaagacgcacctgacacctaccactacgttgttagtgagcctctcggtagaaactcctacaaggagagatacctatttgtctaccgtccagatcaggtgtctgctgtggactcttactactatgacgacggttgtgaaccttgtggttcagacaccttcaacagagaaccagctatcgttagatttttctccagattcaccgaggtcagagagttcgccatcgttccattgcacgctgcgcctggagatgcagtggccgaaattgacgctctctatgatgtctacctggacgttcaggaaaaatggggtctagaagatgttatgctgatgggagacttcaacgctggttgctcttacgttaggccatctcaatggtcaagcatcagactatggacttccccaacgttccaatggcttattcctgactccgctgatactaccgccactcccactcattgtgcatatgacagaattgttgtcgctggtatgctactgcgtggagctgtcgtaccagattctgctctgccatttaacttccaagccgcatatggtctttctgaccaactggctcaagccatctctgatcactaccctgtggaagttatgcttaag

SEQ ID NO: 23 - protein, 282 aa, synthetic construct
  REGION 1..282: note = Artificial synthetic polypeptide sequence
MRGMKLLGALLALAALLQGAVSLKIAAFNIRTFGETKMSSATLVSYIVQILSRYDIALVQEVRDSHLTAVGKLLDNLNQDAPDTYHYVVSEPLGRNSYKERYLFVYRPDQVSAVDSYYYDDGCEPCGSDTFNREPFIVRFFSRFTEVREFAIVPLHAAPGDAVAEIDALYDVYLDVQEKWGLEDVMLMGDFNAGCSYVRPSQWSSIRLWTSPTFQWLIPDSADTTAKPTHCAYDRIVVAGMLLRGAVVPDSALPFNFQAAYGLSDQLAQAISDHYPVEVMLK

SEQ ID NO: 24 - DNA, 846 bp, synthetic construct
  misc_feature 1..846: note = Artificial synthetic polynucleotide sequence
  source 1..846: mol_type = other DNA
atgagaggtatgaagctccttggtgccctcctggctctcgctgctctcctccaaggagcagtttctctaaagattgctgctttcaatattagaacctttggcgagactaaaatgtcctcggcaacattagtatcttacattgttcagatcctttctcgttacgacatagctttggtccaggaggttagagactcccacttgactgccgtcggtaagctgctagacaatcttaaccaagacgcacctgacacctaccactacgttgttagtgagcctctcggtagaaactcctacaaggagagatacctatttgtctaccgtccagatcaggtgtctgctgtggactcttactactatgacgacggttgtgaaccttgtggttcagacaccttcaacagagaaccattcatcgttagatttttctccagattcaccgaggtcagagagttcgccatcgttccattgcacgctgcgcctggagatgcagtggccgaaattgacgctctctatgatgtctacctggacgttcaggaaaaatggggtctagaagatgttatgctgatgggagacttcaacgctggttgctcttacgttaggccatctcaatggtcaagcatcagactatggacttccccaacgttccaatggcttattcctgactccgctgatactaccgccaagcccactcattgtgcatatgacagaattgttgtcgctggtatgctactgcgtggagctgtcgtaccagattctgctctgccatttaacttccaagccgcatatggtctttctgaccaactggctcaagccatctctgatcactaccctgtggaagttatgcttaag

SEQ ID NO: 25 - DNA, 915 bp, synthetic construct
  misc_feature 1..915: note = Artificial synthetic polynucleotide sequence
  source 1..915: mol_type = other DNA
atgtctagagagcttgctccactcctcctactccttcttagtatccactctgcactcgccatgagaatttgtagcttcaatgtaagatccttcggtgaatctaagcaggaggacaaaaacgctatggacgttattgtgaaggtcattaagagatgtgatatcattctagttatggagatcaaggactctaacaacagaatttgccccatccttatggaaaagctgaatagaaactctagaagaggaattacttacaactacgttatctcttctaggctgggtagaaacacttacaaggagcaatatgcatttctatacaaggaaaagctagtttccgttaagcgttcttaccactatcatgactaccaagacggcgatgctgacgttttctccagagaaccattcgttgtttggtttcagtctcctcacaccgctgttaaggacttcgtgattatcccactacacactacgccagaaacctctgtcaaggaaatagatgaacttgttgaagtttacaccgacgtgaagcacagatggaaggccgagaatttcattttcatgggtgatttcaacgccggatgctcatatgtccctaaaaaggcttggaaaaacatccgtttgagaaccgatcctagatttgtctggctcatcggtgaccaagaggacaccacagtcaaaaagtctaccaactgtgcttacgacagaattgttctgcgtggtcaggagattgtttcatctgttgtcccaaagtccaactccgtctttgatttccaaaaggcttacaaactgactgaggaggaagctttagacgtgtccgaccacttccctgtagagtttaagctgcaatcctccagagcattcactaactctaaaaagtcagtcactttgcgtaaaaagactaagtctaagagatcg

SEQ ID NO: 26 - DNA, 846 bp, synthetic construct
  misc_feature 1..846: note = Artificial synthetic polynucleotide sequence
  source 1..846: mol_type = other DNA
atgtctagagagcttgctccactcctcctactccttcttagtatccactctgcactcgccatgagaatttgtagcttcaatgtaagatccttcggtgaatctaagcaggaggacaaaaacgctatggacgttattgtgaaggtcattaagagatgtgatatcattctagttatggagatcaaggactctaacaacagaatttgccccatccttatggaaaagctgaatagaaactctagaagaggaattacttacaactacgttatctcttctaggctgggtagaaacacttacaaggagcaatatgcatttctatacaaggaaaagctagtttccgttaagcgttcttaccactatcatgactaccaagacggcgatgctgacgttttctccagagaaccattcgttgtttggtttcagtctcctcacaccgctgttaaggacttcgtgattatcccactacacactacgccagaaacctctgtcaaggaaatagatgaacttgttgaagtttacaccgacgtgaagcacagatggaaggccgagaatttcattttcatgggtgatttcaacgccggatgctcatatgtccctaaaaaggcttggaaaaacatccgtttgagaaccgatcctagatttgtctggctcatcggtgaccaagaggacaccacagtcaaaaagtctaccaactgtgcttacgacagaattgttctgcgtggtcaggagattgtttcatctgttgtcccaaagtccaactccgtctttgatttccaaaaggcttacaaactgactgaggaggaagctttagacgtgtccgaccactaccctgtagaggtcatgttgaag

SEQ ID NO: 27 - DNA, 20 bp, synthetic construct
  misc_feature 1..20: note = Artificial synthetic polynucleotide sequence
  source 1..20: mol_type = other DNA
gtcgacatgcggtacacagg

SEQ ID NO: 28 - DNA, 26 bp, synthetic construct
  misc_feature 1..26: note = Artificial synthetic polynucleotide sequence
  source 1..26: mol_type = other DNA
ctcgagtcagatttttctgagtgtca

SEQ ID NO: 29 - DNA, 24 bp, synthetic construct
  misc_feature 1..24: note = Artificial synthetic polynucleotide sequence
  source 1..24: mol_type = other DNA
gaagtcccaggaattcaaagatgt

SEQ ID NO: 30 - DNA, 22 bp, synthetic construct
  misc_feature 1..22: note = Artificial synthetic polynucleotide sequence
  source 1..22: mol_type = other DNA
gcgtgatacccgggagcgattg

SEQ ID NO: 31 - DNA, 29 bp, synthetic construct
  misc_feature 1..29: note = Artificial synthetic polynucleotide sequence
  source 1..29: mol_type = other DNA
agtcgactcccggccaccatgtccctgca

SEQ ID NO: 32 - DNA, 29 bp, synthetic construct
  misc_feature 1..29: note = Artificial synthetic polynucleotide sequence
  source 1..29: mol_type = other DNA
tgcagggacatggtggccgggagtcgact

SEQ ID NO: 33 - protein, 23 aa, synthetic construct
  REGION 1..23: note = Artificial synthetic polypeptide sequence
SSRAFTNSKKSVTLRKKTKSKRS

SEQ ID NO: 34 - protein, 310 aa, synthetic construct
  REGION 1..310: note = Artificial synthetic polypeptide sequence
MSLHPASPRLASLLLFILALHDTLALRLCSFNVRSFGASKKENHEAMDIIVKIIKRCDLILLMEIKDSSNNICPMLMEKLNGNSRRSTTYNYVISSRLGRNTYKEQYAFVYKEKLVSVKTKYHYHDYQDGDTDVFSREPFVVWFHSPFTAVKDFVIVPLHTTPETSVKEIDELVDVYTDVRSQWKTENFIFMGDFNAGCSYVPKKAWQNIRLRTDPKFVWLIGDQEDTTVKKSTSCAYDRIVLCGQEIVNSVVPRSSGVFDFQKAYDLSEEEALDVSDHFPVEFKLQSSRAFTNNRKSVSLKKRKKGNRS

SEQ ID NO: 35 - protein, 310 aa, Mus musculus
MSLYPASPYLASLLLFILALHGALSLRLCSFNVRSFGESKKENHNAMDIIVKIIKRCDLILLMEIKDSNNNICPMLMEKLNGNSRRSTTYNYVISSRLGRNTYKEQYAFLYKEKLVSVKAKYLYHDYQDGDTDVFSREPFVVWFQAPFTAAKDFVIVPLHTTPETSVKEIDELADVYTDVRRRWKAENFIFMGDFNAGCSYVPKKAWKNIRLRTDPNFVWLIGDQEDTTVKKSTSCAYDRIVLRGQEIVNSVVPRSSGVFDFQKAYELSEEEALDVSDHFPVEFKLQSSRAFTNSRKSVSLKKKKKGSRS

SEQ ID NO: 36 - protein, 282 aa, synthetic construct
  REGION 1..282: note = Artificial synthetic polypeptide sequence
MRSMKLLGALLALAALLQGAVSLKIAAFNIQTFGETKMSNATLVSYIVQILSRYDIALVQEVRDSHLTAVGKLLDNLNQDAPDTYHYVVSEPLGRNSYKERYLFVYRPDQVSAVDSYYYDDGCEPCGNDTFNREPAIVRFFSRFTEVREFAIVPLHAAPGDAVAEIDALYDVYLDVQEKWGLEDVMLMGDFNAGCSYVRPSQWSSIRLRTSPAFQWLIPDSADTTATPTHCAYDRIVVAGMLLQGAVVPDSALPFNFQAAYGLSDQLAQAISDHYPVEVMLK

SEQ ID NO: 37 - protein, 305 aa, synthetic construct
  REGION 1..305: note = Artificial synthetic polypeptide sequence
MSRELTPLLLLLLSIHSTLALRICSFNVRSFGESKQEDQNAMDVIVKVIKRCDIILVMEIKDSNNRICPILMEKLNRNSRRGITYNYVISSRLGRNTYKEQYAFLYKEKLVSVKRSYHYHDYQDGDADVFSREPFVVWFQSPHTAVKDFVIIPLHTTPETSVKEIDELVEVYTDVKHRWKAENFIFMGDFNAGCSYVPKKAWKNIRLRTDPRFVWLIGDQEDTTVKKSTNCAYDRIVLRGQEIVSSVVPKSNSVFDFQKAYKLTEEEALDVSDHFPVEFKLQSSRAFTNSKKSVTLRKKTKSKRS

SEQ ID NO: 38 - protein, 302 aa, Homo sapiens
MHYPTALLFLILANGAQAFRICAFNAQRLTLAKVAREQVMDTLVRILARCDIMVLQEVVDSSGSAIPLLLRELNRFDGSGPYSTLSSPQLGRSTYMETYVYFYRSHKTQVLSSYVYNDEDDVFAREPFVAQFSLPSNVLPSLVLVPLHTTPKAVEKELNALYDVFLEVSQHWQSKDVILLGDFNADCASLTKKRLDKLELRTEPGFHWVIADGEDTTVRASTHCTYDRVVLHGERCRSLLHTAAAFDFPTSFQLTEEEALNISDHYPVEVELKLSQAHSVQPLSLTVLLLLSLLSPQLCPAA

SEQ ID NO: 39 - protein, 299 aa, Homo sapiens
MGGPRALLAALWALEAAGTAALRIGAFNIQSFGDSKVSDPACGSIIAKILAGYDLALVQEVRDPDLSAVSALMEQINSVSEHEYSFVSSQPLGRDQYKEMYLFVYRKDAVSVVDTYLYPDPEDVFSREPFVVKFSAPGTGERAPPLPSRRALTPPPLPAAAQNLVLIPLHAAPHQAVAEIDALYDVYLDVIDKWGTDDMLFLGDFNADCSYVRAQDWAAIRLRSSEVFKWLIPDSADTTVGNSDCAYDRIVACGARLRRSLKPQSATVHDFQEEFGLDQTQALAISDHFPVEVTLKFHR

SEQ ID NO: 40 - protein, 24 aa, synthetic construct
  REGION 1..24: note = Artificial synthetic polypeptide sequence
QSSRAFTNSKKSVTLRKKTKSKRS